European Patent Specification EP 3 219 805 B1, published January 17, 2024. Title: Method of producing cis-5-hydroxy-L-pipecolic acid. Applicant: API Corporation. The sequence listing filed with the application follows.

SEQUENCE LISTING (13 sequences)

SEQ ID NO: 1 - DNA, 882 bp, Artifical Sequence
  xdph_Ecodon
atgatgagcgcaaaactgctggcaagcattgaattgaaccaagaacagatcgagcatgatctgaatattgttggtagcgagatcctggacgtggcgtacagcgagtatgcgtgcggcaattggggtaccattaccctgtggaaccacagcggcgatgctggcgaccagacgagccgcgaatacgttggtcaggcccgtccgactgagctgggccagcaattagactgcattaatcagctgatccgtaacaatttcaacatcagcctgatcaagagcgtgcgcatcttccgtagctataacggtggtgcgatctatccgcacattgactacttggaattcaaccaaggttttaagcgcgtgcacctggttctgaaatccgaccgttcatgtctgaatagcgaagagaacacggtttatcacatgctgcctggtgaagtgtggtttgtcgatggtcatagcgcgcactcggcgatgagcctgagccgtgtcggcaagtactcgctggtcctggactttgattctggcgccaaattcgaagatctgtattctgagagccacaccctgtgtgttgataacctggagccggacattatccatgaccgccagccactgccgaccagcctgcgtgatagcctggcacacattgctgagcatgcggatgaattcaatatccaatccattctgttcctggccacccgttttcactttagctacgcagtgagcattcgtgagtacttccaactcctggacgagtgcttttctcgcaacccgtacaagtccgttcgcgagcgttacgaagcgctgaaagacattttggtgcgtagcggttataccagccacaatgtcaatcatttcaacagcttgtccggtgtcacgatcggc

SEQ ID NO: 2 - DNA, 843 bp, Artifical Sequence
  smph_Ecodon
atgagcacccattttctcggcaaggtaaagtttgatgaagcgcgtttggcagaggacttgagcaccctggaagtggctgagtttagcagcgcctacagcgactttgcatgcggcaaatgggaagcgtgcgtcctgcgcaaccgcaccggtatgcaagaagaagatatcgttgttagccacaatgctccggcgctggcgacgccgctgagcaagtccctgccgtatctgaacgagctggtggaaacccatttcgactgtagcgccgtgcgttacacgcgcattgttcgtgtctctgagaacgcatgtatcattccgcattctgactatctggagttggatgaaacgttcacgcgcctgcacctggttctggacacgaatagcggttgtgcgaataccgaagaggataagattttccacatgggtctgggcgagatctggttcctggatgctatgctgccgcacagcgccgcatgctttagcaaaactccgcgtctgcacttgatgattgatttcgaggcgaccgcgttcccagagagctttttgcgtaacgttgagcagccggtcaccacccgtgatatggtggacccgcgtaaagagctgaccgacgaggtgatcgaaggtatcctgggcttttccatcatcattagcgaggcaaattaccgtgagattgtctccattctggcgaaactgcacttcttttacaaggcggattgccgcagcatgtacgactggctgaaagaaatctgcaaacgtcgtggtgaccctgccctgattgaaaagaccgcgtcgctggagcgcttcttcctgggtcatcgtgaacgcggtgaggttatgacgtattaa

SEQ ID NO: 3 - DNA, 897 bp, Artifical Sequence
  sruph_Ecodon
atgaaaagctattccttgggcaagtttgaggaccgttctattgacagcctgatcgaagaagcgtccggtctgccggacagcgcgtattcttctgcgtaccaagagtacagcatcggtctgtgggacaccgccacgctgtggaacgaacgtggcaacgagagcggcgaggttagcgagcacgcggcagccgctgcgccgaccgcaattggtcgtagcaccccgcgtctgaacgaatttgtacgtgccaagttcaatgtcgatgtcctgcgtgcggttcgcttgttcagagcgcgtcagggtgcaattatcatcccgcaccgcgattacctggagcatagcaatggtttttgccgtattcaccttccgctggttacgaccccgggtgcgcgtaatagcgagaataacgaagtgtatcgcatgctgcctggcgagctgtggttcctggattcaaacgaagtgcacagcggtggcgttctggacagcggtacgcgcattcacctcgttttagatttcacccacgagcataatgagaatccggctgcagtgctgaagaacgccgaccgtttgcgtccgatcgcgcgtgacccgcgcatctcgcgctccaaactggatcacgaagcgctggagagcctgatccgcggtggccgtgtcgtcactctggcgatgtggccagctctggtgcagatgctggcacgcattcatctgaccagcgacgcacatccggccgagctgtacgactggttggatgacctggcggaccgcagcggcaacgatgagctggttgcagaagcgcgtcgtatgcgtcgttactttctgaccgatggtattagccgtacgccgagcttcgaacgcttttggcgcgaactggatgccgctcgtaaaggtgagttggtgagc

SEQ ID NO: 4 - protein, 294 aa, Xenorhabdus doucetiae FRM16
MMSAKLLASIELNQEQIEHDLNIVGSEILDVAYSEYACGNWGTITLWNHSGDAGDQTSREYVGQARPTELGQQLDCINQLIRNNFNISLIKSVRIFRSYNGGAIYPHIDYLEFNQGFKRVHLVLKSDRSCLNSEENTVYHMLPGEVWFVDGHSAHSAMSLSRVGKYSLVLDFDSGAKFEDLYSESHTLCVDNLEPDIIHDRQPLPTSLRDSLAHIAEHADEFNIQSILFLATRFHFSYAVSIREYFQLLDECFSRNPYKSVRERYEALKDILVRSGYTSHNVNHFNSLSGVTIG

SEQ ID NO: 5 - protein, 280 aa, Sinorhizobium meliloti 1021 [sequence omitted]

SEQ ID NO: 6 - protein, 299 aa, Segniliparus rugosus ATCC BAA-974
MKSYSLGKFEDRSIDSLIEEASGLPDSAYSSAYQEYSIGLWDTATLWNERGNESGEVSEHAAAAAPTAIGRSTPRLNEFVRAKFNVDVLRAVRLFRARQGAIIIPHRDYLEHSNGFCRIHLPLVTTPGARNSENNEVYRMLPGELWFLDSNEVHSGGVLDSGTRIHLVLDFTHEHNENPAAVLKNADRLRPIARDPRISRSKLDHEALESLIRGGRVVTLAMWPALVQMLARIHLTSDAHPAELYDWLDDLADRSGNDELVAEARRMRRYFLTDGISRTPSFERFWRELDAARKGELVS

SEQ ID NO: 7 - DNA, 36 bp, Artifical Sequence
  primer
tttcatatgagcacccattttctcggcaaggtaaag

SEQ ID NO: 8 - DNA, 33 bp, Artifical Sequence
  primer
tttaagcttttaatacgtcataacctcaccgcg

SEQ ID NO: 9 - DNA, 858 bp, Xenorhabdus doucetiae FRM16
atgagaacgcattttgtgggtgaagttgcattggacctggcacgtctggaggctgatctggcaacctgtcgtagcctggagtggagcgaagcgtattcggattacgtctttggtggtagctggaaaagctgcatgctgtgggcgcctggtggcgatgccggcgatggtgttgtgacggactacgcgtacgaccgtagcgcgggttttacgccgcacgcagagcgcctgccgtatctggcagagcttattcgtgagactgcagatctggatcgcctgaatttcgcgcgcttggcgctggtaaccaactctgtgattatcccgcaccgtgacctgttggaattaagcgacttgccggacgaagctcgcaatgaacaccgtatgcacattccgctggcgaccaatgataactgcttcttcaacgaggacaacgttgtgtatcgtatgcgtcgtggtgaagtttggtttctggatgccagccgtattcatagcgtcgctgtcctgacggcgcagccacgtatccatctgatgctggatttcgtggacaccccgggtgcgggcagcttcacgcgcgttgcgggtggcggcgttgaggccggcatcccggtcgatcgcatcgtgacccgtccgccgctgggcgacgacgagcgtgcggacctgttcggtgtcgccccactcctgtccatggataccttcgacgaagtgttttccattgttatcaagaaacacttccgtcgtgatggtggcagcgactttgtgtgggacaccatgctggaactggcggcgaagtctccggatccggccgtcctgccgcataccgaagaactgcgcaagcactacaccctggaccgcagcgcataa

SEQ ID NO: 10 - DNA, 885 bp, Xenorhabdus romanii PR06-A
atgatgagtgcaaaattgttggccagcattgaactgaatcaggaacaaattgaacacgacttaaatattgtaggtagtgaaattctggatgttgcatatagcgaatatgcttgtggcaactggggcaccatcacgttatggaatcacagtggagacgctggtgaccaaacatcaagagagtatgttgggcaggctcgtcctacagagcttggacagcagttggattgtattaaccaacttattcgaaacaattttaatatatctctgatcaaatcagtgcgtatattccgttcttataacggtggagccatttatccacatattgattatttggaattcaatcaagggttcaaacgtgtgcatctggtgctaaaatcagaccgaagttgcctcaattccgaagagaatacagtttatcacatgctccctggtgaagtatggtttgttgacggtcatagtgcacacagtgcaatgtcactaagtcgtgtagggaaatacagtttagtgcttgattttgactctggtgctaaattcgaggatttgtattccgaaagccacacgttatgtgtagacaacctagaaccagatattattcatgatcggcaaccattgccaacatcactgcgggattcactcgctcatatagctgagcacgccgatgaattcaacattcagtctatcctgtttcttgctacccgctttcactttagttatgcagtgtcaatcagagaatattttcaattgttagatgaatgttttagtcgtaatccgtacaaatcagttagagaaagatacgaggcattgaaggatattctagtccgaagtggctatacatcccataagtttaaccactttaactcactgtctggagtcactattggttaa

SEQ ID NO: 11 - protein, 294 aa, Xenorhabdus romanii PR06-A
MMSAKLLASIELNQEQIEHDLNIVGSEILDVAYSEYACGNWGTITLWNHSGDAGDQTSREYVGQARPTELGQQLDCINQLIRNNFNISLIKSVRIFRSYNGGAIYPHIDYLEFNQGFKRVHLVLKSDRSCLNSEENTVYHMLPGEVWFVDGHSAHSAMSLSRVGKYSLVLDFDSGAKFEDLYSESHTLCVDNLEPDIIHDRQPLPTSLRDSLAHIAEHADEFNIQSILFLATRFHFSYAVSIREYFQLLDECFSRNPYKSVRERYEALKDILVRSGYTSHKFNHFNSLSGVTIG

SEQ ID NO: 12 - DNA, 47 bp, Artificial Sequence
  primer
gaattcattaaagaggagaaattaaccatgatgagtgcaaaattgtt

SEQ ID NO: 13 - DNA, 47 bp, Artificial Sequence
  primer
caacaggagtccaagctcagctaattattaaccaatagtgactccag